European Patent Specification EP 3 934 673 B1, published January 7, 2026. Title: SYNTHETIC ONCOLYTIC LNP-REPLICON RNA FOR CANCER IMMUNOTHERAPY. Applicant: Massachusetts Institute of Technology. Application Not Yet Assigned. The sequence listing filed with the application follows.

SEQUENCE LISTING (5 sequences)

SEQ ID NO: 1 - DNA, 10276 bp, Unknown
  VEE virus
atgggcggcgcatgagagaagcccagaccaattacctacccaaaatggagaaagttcacgttgacatcgaggaagacagcccattcctcagagctttgcagcggagcttcccgcagtttgaggtagaagccaagcaggtcactgataatgaccatgctaatgccagagcgttttcgcatctggcttcaaaactgatcgaaacggaggtggacccatccgacacgatccttgacattggaagtgcgcccgcccgcagaatgtattctaagcacaagtatcattgtatctgtccgatgagatgtgcggaagatccggacagattgtataagtatgcaactaagctgaagaaaaactgtaaggaaataactgataaggaattggacaagaaaatgaaggagctggccgccgtcatgagcgaccctgacctggaaactgagactatgtgcctccacgacgacgagtcgtgtcgctacgaagggcaagtcgctgtttaccaggatgtatacgcggttgacggaccgacaagtctctatcaccaagccaataagggagttagagtcgcctactggataggctttgacaccaccccttttatgtttaagaacttggctggagcatatccatcatactctaccaactgggccgacgaaaccgtgttaacggctcgtaacataggcctatgcagctctgacgttatggagcggtcacgtagagggatgtccattcttagaaagaagtatttgaaaccatccaacaatgttctattctctgttggctcgaccatctaccacgagaagagggacttactgaggagctggcacctgccgtctgtatttcacttacgtggcaagcaaaattacacatgtcggtgtgagactatagttagttgcgacgggtacgtcgttaaaagaatagctatcagtccaggcctgtatgggaagccttcaggctatgctgctacgatgcaccgcgagggattcttgtgctgcaaagtgacagacacattgaacggggagagggtctcttttcccgtgtgcacgtatgtgccagctacattgtgtgaccaaatgactggcatactggcaacagatgtcagtgcggacgacgcgcaaaaactgctggttgggctcaaccagcgtatagtcgtcaacggtcgcacccagagaaacaccaataccatgaaaaattaccttttgcccgtagtggcccaggcatttgctaggtgggcaaaggaatataaggaagatcaagaagatgaaaggccactaggactacgagatagacagttagtcatggggtgttgttgggcttttagaaggcacaagataacatctatttataagcgcccggatacccaaaccatcatcaaagtgaacagcgatttccactcattcgtgctgcccaggataggcagtaacacattggagatcgggctgagaacaagaatcaggaaaatgttagaggagcacaaggagccgtcacctctcattaccgccgaggacgtacaagaagctaagtgcgcagccgatgaggctaaggaggtgcgtgaagccgaggagttgcgcgcagctctaccacctttggcagctgatgttgaggagcccactctggaggcagacgtcgacttgatgttacaagaggctggggccggctcagtggagacacctcgtggcttgataaaggttaccagctacgatggcgaggacaagatcggctcttacgctgtgctttctccgcaggctgtactcaagagtgaaaaattatcttgcatccaccctctcgctgaacaagtcatagtgataacacactctggccgaaaagggcgttatgccgtggaaccataccatggtaaagtagtggtgccagagggacatgcaatacccgtccaggactttcaagctctgagtgaaagtgccaccattgtgtacaacgaacgtgagttcgtaaacaggtacctgcaccatattgccacacatggaggagcgctgaacactgatgaagaatattacaaaactgtcaagcccagcgagcacgacggcgaatacctgtacgacatcgacaggaaacagtgcgtcaagaaagaactagtcactgggctagggctcacaggcgagctggtggatcctcccttccatgaattcgcctacgagagtctgagaacacgaccagccgctccttaccaagtaccaaccataggggtgtatggcgtgccaggatcaggcaagtctggcatcattaaaagcgcagtcaccaaaaaagatctagtggtgagcgccaagaaagaaaactgtgcagaaattataagggacgtcaagaaaatgaaagggctggacgtcaatgccagaactgtggactcagtgctcttgaatggatgcaaacaccccgtagagaccctgtatattgacgaagcttttgcttgtcatgcaggtactctcagagcgctcatagccattataagacctaaaaaggcagtgctctgcggggatcccaaacagtgcggtttttttaacatgatgtgcctgaaagtgcattttaaccacgagatttgcacacaagtcttccacaaaagcatctctcgccgttgcactaaatctgtgacttcggtcgtctcaaccttgttttacgacaaaaaaatgagaacgacgaatccgaaagagactaagattgtgattgacactaccggcagtaccaaacctaagcaggacgatctcattctcacttgtttcagagggtgggtgaagcagttgcaaatagattacaaaggcaacgaaataatgacggcagctgcctctcaagggctgacccgtaaaggtgtgtatgccgttcggtacaaggtgaatgaaaatcctctgtacgcacccacctcagaacatgtgaacgtcctactgacccgcacggaggaccgcatcgtgtggaaaacactagccggcgacccatggataaaaacactgactgccaagtaccctgggaatttcactgccacgatagaggagtggcaagcagagcatgatgccatcatgaggcacatcttggagagaccggaccctaccgacgtcttccagaataaggcaaacgtgtgttgggccaaggctttagtgccggtgctgaagaccgctggcatagacatgaccactgaacaatggaacactgtggattattttgaaacggacaaagctcactcagcagagatagtattgaaccaactatgcgtgaggttctttggactcgatctggactccggtctattttctgcacccactgttccgttatccattaggaataatcactgggataactccccgtcgcctaacatgtacgggctgaataaagaagtggtccgtcagctctctcgcaggtacccacaactgcctcgggcagttgccactggaagagtctatgacatgaacactggtacactgcgcaattatgatccgcgcataaacctagtacctgtaaacagaagactgcctcatgctttagtcctccaccataatgaacacccacagagtgacttttcttcattcgtcagcaaattgaagggcagaactgtcctggtggtcggggaaaagttgtccgtcccaggcaaaatggttgactggttgtcagaccggcctgaggctaccttcagagctcggctggatttaggcatcccaggtgatgtgcccaaatatgacataatatttgttaatgtgaggaccccatataaataccatcactatcagcagtgtgaagaccatgccattaagcttagcatgttgaccaagaaagcttgtctgcatctgaatcccggcggaacctgtgtcagcataggttatggttacgctgacagggccagcgaaagcatcattggtgctatagcgcggcagttcaagttttcccgggtatgcaaaccgaaatcctcacttgaagagacggaagttctgtttgtattcattgggtacgatcgcaaggcccgtacgcacaattcttacaagctttcatcaaccttgaccaacatttatacaggttccagactccacgaagccggatgtgcaccctcatatcatgtggtgcgaggggatattgccacggccaccgaaggagtgattataaatgctgctaacagcaaaggacaacctggcggaggggtgtgcggagcgctgtataagaaattcccggaaagcttcgatttacagccgatcgaagtaggaaaagcgcgactggtcaaaggtgcagctaaacatatcattcatgccgtaggaccaaacttcaacaaagtttcggaggttgaaggtgacaaacagttggcagaggcttatgagtccatcgctaagattgtcaacgataacaattacaagtcagtagcgattccactgttgtccaccggcatcttttccgggaacaaagatcgactaacccaatcattgaaccatttgctgacagctttagacaccactgatgcagatgtagccatatactgcagggacaagaaatgggaaatgactctcaaggaagcagtggctaggagagaagcagtggaggagatatgcatatccgacgactcttcagtgacagaacctgatgcagagctggtgagggtgcatccgaagagttctttggctggaaggaagggctacagcacaagcgatggcaaaactttctcatatttggaagggaccaagtttcaccaggcggccaaggatatagcagaaattaatgccatgtggcccgttgcaacggaggccaatgagcaggtatgcatgtatatcctcggagaaagcatgagcagtattaggtcgaaatgccccgtcgaagagtcggaagcctccacaccacctagcacgctgccttgcttgtgcatccatgccatgactccagaaagagtacagcgcctaaaagcctcacgtccagaacaaattactgtgtgctcatcctttccattgccgaagtatagaatcactggtgtgcagaagatccaatgctcccagcctatattgttctcaccgaaagtgcctgcgtatattcatccaaggaagtatctcgtggaaacaccaccggtagacgagactccggagccatcggcagagaaccaatccacagaggggacacctgaacaaccaccacttataaccgaggatgagaccaggactagaacgcctgagccgatcatcatcgaagaggaagaagaggatagcataagtttgctgtcagatggcccgacccaccaggtgctgcaagtcgaggcagacattcacgggccgccctctgtatctagctcatcctggtccattcctcatgcatccgactttgatgtggacagtttatccatacttgacaccctggagggagctagcgtgaccagcggggcaacgtcagccgagactaactcttacttcgcaaagagtatggagtttctggcgcgaccggtgcctgcgcctcgaacagtattcaggaaccctccacatcccgctccgcgcacaagaacaccgtcacttgcacccagcagggcctgctcgagaaccagcctagtttccaccccgccaggcgtgaatagggtgatcactagagaggagctcgaggcgcttaccccgtcacgcactcctagcaggtcggtctcgagaaccagcctggtctccaacccgccaggcgtaaatagggtgattacaagagaggagtttgaggcgttcgtagcacaacaacaatgacggtttgatgcgggtgcatacatcttttcctccgacaccggtcaagggcatttacaacaaaaatcagtaaggcaaacggtgctatccgaagtggtgttggagaggaccgaattggagatttcgtatgccccgcgcctcgaccaagaaaaagaagaattactacgcaagaaattacagttaaatcccacacctgctaacagaagcagataccagtccaggaaggtggagaacatgaaagccataacagctagacgtattctgcaaggcctagggcattatttgaaggcagaaggaaaagtggagtgctaccgaaccctgcatcctgttcctttgtattcatctagtgtgaaccgtgccttttcaagccccaaggtcgcagtggaagcctgtaacgccatgttgaaagagaactttccgactgtggcttcttactgtattattccagagtacgatgcctatttggacatggttgacggagcttcatgctgcttagacactgccagtttttgccctgcaaagctgcgcagctttccaaagaaacactcctatttggaacccacaatacgatcggcagtgccttcagcgatccagaacacgctccagaacgtcctggcagctgccacaaaaagaaattgcaatgtcacgcaaatgagagaattgcccgtattggattcggcggcctttaatgtggaatgcttcaagaaatatgcgtgtaataatgaatattgggaaacgtttaaagaaaaccccatcaggcttactgaagaaaacgtggtaaattacattaccaaattaaaaggaccaaaagctgctgctctttttgcgaagacacataatttgaatatgttgcaggacataccaatggacaggtttgtaatggacttaaagagagacgtgaaagtgactccaggaacaaaacatactgaagaacggcccaaggtacaggtgatccaggctgccgatccgctagcaacagcgtatctgtgcggaatccaccgagagctggttaggagattaaatgcggtcctgcttccgaacattcatacactgtttgatatgtcggctgaagactttgacgctattatagccgagcacttccagcctggggattgtgttctggaaactgacatcgcgtcgtttgataaaagtgaggacgacgccatggctctgaccgcgttaatgattctggaagacttaggtgtggacgcagagctgttgacgctgattgaggcggctttcggcgaaatttcatcaatacatttgcccactaaaactaaatttaaattcggagccatgatgaaatctggaatgttcctcacactgtttgtgaacacagtcattaacattgtaatcgcaagcagagtgttgagagaacggctaaccggatcaccatgtgcagcattcattggagatgacaatatcgtgaaaggagtcaaatcggacaaattaatggcagacaggtgcgccacctggttgaatatggaagtcaagattatagatgctgtggtgggcgagaaagcgccttatttctgtggagggtttattttgtgtgactccgtgaccggcacagcgtgccgtgtggcagaccccctaaaaaggctgtttaagcttggcaaacctctggcagcagacgatgaacatgatgatgacaggagaagggcattgcatgaagagtcaacacgctggaaccgagtgggtattctttcagagctgtgcaaggcagtagaatcaaggtatgaaaccgtaggaacttccatcatagttatggccatgactactctagctagcagtgttaaatcattcagctacctgagaggggcccctataactctctacggctaacctgaatggactacgacatagtctagtccgccaagtctagcatatgggcgcgccctcagcatcgattgaattggccaccatggtgagcaagggcgaggaggataacatggccatcatcaaggagttcatgcgcttcaaggtgcacatggagggctccgtgaacggccacgagttcgagatcgagggcgagggcgagggccgcccctacgagggcacccagaccgccaagctgaaggtgaccaagggtggccccctgcccttcgcctgggacatcctgtcccctcagttcatgtacggctccaaggcctacgtgaagcaccccgccgacatccccgactacttgaagctgtccttccccgagggcttcaagtgggagcgcgtgatgaacttcgaggacggcggcgtggtgaccgtgacccaggactcctccctgcaggacggcgagttcatctacaaggtgaagctgcgcggcaccaacttcccctccgacggccccgtaatgcagaagaagaccatgggctgggaggcctcctccgagcggatgtaccccgaggacggcgccctgaagggcgagatcaagcagaggctgaagctgaaggacggcggccactacgacgctgaggtcaagaccacctacaaggccaagaagcccgtgcagctgcccggcgcctacaacgtcaacatcaagttggacatcacctcccacaacgaggactacaccatcgtggaacagtacgaacgcgccgagggccgccactccaccggcggcatggacgagctgtacaagtaggaattggcaagctgcttacatagaactcgcggcgattggcatgccgccttaaaatttttattttatttttcttttcttttccgaatcggattttgtttttaatatttcaaaaaaaaaaaaaaaaaaaaaaaaaacgcgtcgaggggaattaattcttgaagacgaaagggccaggtggcacttttcggggaaatgtgcgcggaacccctatttgtttatttttctaaatacattcaaatatgtatccgctcatgagacaataaccctgataaatgcttcaataatattgaaaaaggaagagtatgagtattcaacatttccgtgtcgcccttattcccttttttgcggcattttgccttcctgtttttgctcacccagaaacgctggtgaaagtaaaagatgctgaagatcagttgggtgcacgagtgggttacatcgaactggatctcaacagcggtaagatccttgagagttttcgccccgaagaacgttttccaatgatgagcacttttaaagttctgctatgtggcgcggtattatcccgtgttgacgccgggcaagagcaactcggtcgccgcatacactattctcagaatgacttggttgagtactcaccagtcacagaaaagcatcttacggatggcatgacagtaagagaattatgcagtgctgccataaccatgagtgataacactgcggccaacttacttctgacaacgatcggaggaccgaaggagctaaccgcttttttgcacaacatgggggatcatgtaactcgccttgatcgttgggaaccggagctgaatgaagccataccaaacgacgagcgtgacaccacgatgcctgtagcaatggcaacaacgttgcgcaaactattaactggcgaactacttactctagcttcccggcaacaattaatagactggatggaggcggataaagttgcaggaccacttctgcgctcggcccttccggctggctggtttattgctgataaatctggagccggtgagcgtgggtctcgcggtatcattgcagcactggggccagatggtaagccctcccgtatcgtagttatctacacgacggggagtcaggcaactatggatgaacgaaatagacagatcgctgagataggtgcctcactgattaagcattggtaactgtcagaccaagtttactcatatatactttagattgatttaaaacttcatttttaatttaaaaggatctaggtgaagatcctttttgataatctcatgaccaaaatcccttaacgtgagttttcgttccactgagcgtcagaccccgtagaaaagatcaaaggatcttcttgagatcctttttttctgcgcgtaatctgctgcttgcaaacaaaaaaaccaccgctaccagcggtggtttgtttgccggatcaagagctaccaactctttttccgaaggtaactggcttcagcagagcgcagataccaaatactgtccttctagtgtagccgtagttaggccaccacttcaagaactctgtagcaccgcctacatacctcgctctgctaatcctgttaccagtggctgctgccagtggcgataagtcgtgtcttaccgggttggactcaagacgatagttaccggataaggcgcagcggtcgggctgaacggggggttcgtgcacacagcccagcttggagcgaacgacctacaccgaactgagatacctacagcgtgagcattgagaaagcgccacgcttcccgaagggagaaaggcggacaggtatccggtaagcggcagggtcggaacaggagagcgcacgagggagcttccagggggaaacgcctggtatctttatagtcctgtcgggtttcgccacctctgacttgagcgtcgatttttgtgatgctcgtcaggggggcggagcctatggaaaaacgccagcaacgcgagctctaatacgactcactatag

SEQ ID NO: 2 - DNA, 10276 bp, Artificial Sequence
  Synthetic polynucleotide
atgggcggcgcatgagagaagcccagaccaattacctacccaaaatggagaaagttcacgttgacatcgaggaagacagcccattcctcagagctttgcagcggagcttcccgcagtttgaggtagaagccaagcaggtcactgataatgaccatgctaatgccagagcgttttcgcatctggcttcaaaactgatcgaaacggaggtggacccatccgacacgatccttgacattggaagtgcgcccgcccgcagaatgtattctaagcacaagtatcattgtatctgtccgatgagatgtgcggaagatccggacagattgtataagtatgcaactaagctgaagaaaaactgtaaggaaataactgataaggaattggacaagaaaatgaaggagctggccgccgtcatgagcgaccctgacctggaaactgagactatgtgcctccacgacgacgagtcgtgtcgctacgaagggcaagtcgctgtttaccaggatgtatacgcggttgacggaccgacaagtctctatcaccaagccaataagggagttagagtcgcctactggataggctttgacaccaccccttttatgtttaagaacttggctggagcatatccatcatactctaccaactgggccgacgaaaccgtgttaacggctcgtaacataggcctatgcagctctgacgttatggagcggtcacgtagagggatgtccattcttagaaagaagtatttgaaaccatccaacaatgttctattctctgttggctcgaccatctaccacgagaagagggacttactgaggagctggcacctgccgtctgtatttcacttacgtggcaagcaaaattacacatgtcggtgtgagactatagttagttgcgacgggtacgtcgttaaaagaatagctatcagtccaggcctgtatgggaagccttcaggctatgctgctacgatgcaccgcgagggattcttgtgctgcaaagtgacagacacattgaacggggagagggtctcttttcccgtgtgcacgtatgtgccagctacattgtgtgaccaaatgactggcatactggcaacagatgtcagtgcggacgacgcgcaaaaactgctggttgggctcaaccagcgtatagtcgtcaacggtcgcacccagagaaacaccaataccatgaaaaattaccttttgcccgtagtggcccaggcatttgctaggtgggcaaaggaatataaggaagatcaagaagatgaaaggccactaggactacgagatagacagttagtcatggggtgttgttgggcttttagaaggcacaagataacatctatttataagcgcccggatacccaaaccatcatcaaagtgaacagcgatttccactcattcgtgctgcccaggataggcagtaacacattggagatcgggctgagaacaagaatcaggaaaatgttagaggagcacaaggagccgtcacctctcattaccgccgaggacgtacaagaagctaagtgcgcagccgatgaggctaaggaggtgcgtgaagccgaggagttgcgcgcagctctaccacctttggcagctgatgttgaggagcccactctggaggcagacgtcgacttgatgttacaagaggctggggccggctcagtggagacacctcgtggcttgataaaggttaccagctacgatggcgaggacaagatcggctcttacgctgtgctttctccgcaggctgtactcaagagtgaaaaattatcttgcatccaccctctcgctgaacaagtcatagtgataacacactctggccgaaaagggcgttatgccgtggaaccataccatggtaaagtagtggtgccagagggacatgcaatacccgtccaggactttcaagctctgagtgaaagtgccaccattgtgtacaacgaacgtgagttcgtaaacaggtacctgcaccatattgccacacatggaggagcgctgaacactgatgaagaatattacaaaactgtcaagcccagcgagcacgacggcgaatacctgtacgacatcgacaggaaacagtgcgtcaagaaagaactagtcactgggctagggctcacaggcgagctggtggatcctcccttccatgaattcgcctacgagagtctgagaacacgaccagccgctccttaccaagtaccaaccataggggtgtatggcgtgccaggatcaggcaagtctggcatcattaaaagcgcagtcaccaaaaaagatctagtggtgagcgccaagaaagaaaactgtgcagaaattataagggacgtcaagaaaatgaaagggctggacgtcaatgccagaactgtggactcagtgctcttgaatggatgcaaacaccccgtagagaccctgtatattgacgaagcttttgcttgtcatgcaggtactctcagagcgctcatagccattataagacctaaaaaggcagtgctctgcggggatcccaaacagtgcggtttttttaacatgatgtgcctgaaagtgcattttaaccacgagatttgcacacaagtcttccacaaaagcatctctcgccgttgcactaaatctgtgacttcggtcgtctcaaccttgttttacgacaaaaaaatgagaacgacgaatccgaaagagactaagattgtgattgacactaccggcagtaccaaacctaagcaggacgatctcattctcacttgtttcagagggtgggtgaagcagttgcaaatagattacaaaggcaacgaaataatgacggcagctgcctctcaagggctgacccgtaaaggtgtgtatgccgttcggtacaaggtgaatgaaaatcctctgtacgcacccacctcagaacatgtgaacgtcctactgacccgcacggaggaccgcatcgtgtggaaaacactagccggcgacccatggataaaaacactgactgccaagtaccctgggaatttcactgccacgatagaggagtggcaagcagagcatgatgccatcatgaggcacatcttggagagaccggaccctaccgacgtcttccagaataaggcaaacgtgtgttgggccaaggctttagtgccggtgctgaagaccgctggcatagacatgaccactgaacaatggaacactgtggattattttgaaacggacaaagctcactcagcagagatagtattgaaccaactatgcgtgaggttctttggactcgatctggactccggtctattttctgcacccactgttccgttatccattaggaataatcactgggataactccccgtcgcctaacatgtacgggctgaataaagaagtggtccgtcagctctctcgcaggtacccacaactgcctcgggcagttgccactggaagagtctatgacatgaacactggtacactgcgcaattatgatccgcgcataaacctagtacctgtaaacagaagactgcctcatgctttagtcctccaccataatgaacacccacagagtgacttttcttcattcgtcagcaaattgaagggcagaactgtcctggtggtcggggaaaagttgtccgtcccaggcaaaatggttgactggttgtcagaccggcctgaggctaccttcagagctcggctggatttaggcatcccaggtgatgtgcccaaatatgacataatatttgttaatgtgaggaccccatataaataccatcactatcagcagtgtgaagaccatgccattaagcttagcatgttgaccaagaaagcttgtctgcatctgaatcccggcggaacctgtgtcagcataggttatggttacgctgacagggccagcgaaagcatcattggtgctatagcgcggcagttcaagttttcccgggtatgcaaaccgaaatcctcacttgaagagacggaagttctgtttgtattcattcggtacgatcgcaaggcccgtacgcacaattcttacaagctttcatcaaccttgaccaacatttatacaggttccagactccacgaagccggatgtgcaccctcatatcatgtggtgcgaggggatattgccacggccaccgaaggagtgattataaatgctgctaacagcaaaggacaacctggcggaggggtgtgcggagcgctgtataagaaattcccggaaagcttcgatttacagccgatcgaagtaggaaaagcgcgactggtcaaaggtgcagctaaacatatcattcatgccgtaggaccaaacttcaacaaagtttcggaggttgaaggtgacaaacagttggcagaggcttatgagtccatcgctaagattgtcaacgataacaattacaagtcagtagcgattccactgttgtccaccggcatcttttccgggaacaaagatcgactaacccaatcattgaaccatttgctgacagctttagacaccactgatgcagatgtagccatatactgcagggacaagaaatgggaaatgactctcaaggaagcagtggctaggagagaagcagtggaggagatatgcatatccgacgactcttcagtgacagaacctgatgcagagctggtgagggtgcatccgaagagttctttggctggaaggaagggctacagcacaagcgatggcaaaactttctcatatttggaagggaccaagtttcaccaggcggccaaggatatagcagaaattaatgccatgtggcccgttgcaacggaggccaatgagcaggtatgcatgtatatcctcggagaaggcatgagcagtattaggtcgaaatgccccgtcgaagagtcggaagcctccacaccacctagcacgctgccttgcttgtgcatccatgccatgactccagaaagagtacagcgcctaaaagcctcacgtccagaacaaattactgtgtgctcatcctttccattgccgaagtatagaatcactggtgtgcagaagatccaatgctcccagcctatattgttctcaccgaaagtgcctgcgtatattcatccaaggaagtatctcgtggaaacaccaccggtagacgagactccggagccatcggcagagaaccaatccacagaggggacacctgaacaaccaccacttataaccgaggatgagaccaggactagaacgcctgagccgatcatcatcgaagaggaagaagaggatagcataagtttgctgtcagatggcccgacccaccaggtgctgcaagtcgaggcagacattcacgggccgccctctgtatctagctcatcctggtccattcctcatgcatccgactttgatgtggacagtttatccatacttgacaccctggagggagctagcgtgaccagcggggcaacgtcagccgagactaactcttacttcgcaaagagtatggagtttctggcgcgaccggtgcctgcgcctcgaacagtattcaggaaccctccacatcccgctccgcgcacaagaacaccgtcacttgcacccagcagggcctgctcgagaaccagcctagtttccaccccgccaggcgtgaatagggtgatcactagagaggagctcgaggcgcttaccccgtcacgcactcctagcaggtcggtctcgagaaccagcctggtctccaacccgccaggcgtaaatagggtgattacaagagaggagtttgaggcgttcgtagcacaacaacaatgacggtttgatgcgggtgcatacatcttttcctccgacaccggtcaagggcatttacaacaaaaatcagtaaggcaaacggtgctatccgaagtggtgttggagaggaccgaattggagatttcgtatgccccgcgcctcgaccaagaaaaagaagaattactacgcaagaaattacagttaaatcccacacctgctaacagaagcagataccagtccaggaaggtggagaacatgaaagccataacagctagacgtattctgcaaggcctagggcattatttgaaggcagaaggaaaagtggagtgctaccgaaccctgcatcctgttcctttgtattcatctagtgtgaaccgtgccttttcaagccccaaggtcgcagtggaagcctgtaacgccatgttgaaagagaactttccgactgtggcttcttactgtattattccagagtacgatgcctatttggacatggttgacggagcttcatgctgcttagacactgccagtttttgccctgcaaagctgcgcagctttccaaagaaacactcctatttggaacccacaatacgatcggcagtgccttcagcgatccagaacacgctccagaacgtcctggcagctgccacaaaaagaaattgcaatgtcacgcaaatgagagaattgcccgtattggattcggcggcctttaatgtggaatgcttcaagaaatatgcgtgtaataatgaatattgggaaacgtttaaagaaaaccccatcaggcttactgaagaaaacgtggtaaattacattaccaaattaaaaggaccaaaagctgctgctctttttgcgaagacacataatttgaatatgttgcaggacataccaatggacaggtttgtaatggacttaaagagagacgtgaaagtgactccaggaacaaaacatactgaagaacggcccaaggtacaggtgatccaggctgccgatccgctagcaacagcgtatctgtgcggaatccaccgagagctggttaggagattaaatgcggtcctgcttccgaacattcatacactgtttgatatgtcggctgaagactttgacgctattatagccgagcacttccagcctggggattgtgttctggaaactgacatcgcgtcgtttgataaaagtgaggacgacgccatggctctgaccgcgttaatgattctggaagacttaggtgtggacgcagagctgttgacgctgattgaggcggctttcggcgaaatttcatcaatacatttgcccactaaaactaaatttaaattcggagccatgatgaaatctggaatgttcctcacactgtttgtgaacacagtcattaacattgtaatcgcaagcagagtgttgagagaacggctaaccggatcaccatgtgcagcattcattggagatgacaatatcgtgaaaggagtcaaatcggacaaattaatggcagacaggtgcgccacctggttgaatatggaagtcaagattatagatgctgtggtgggcgagaaagcgccttatttctgtggagggtttattttgtgtgactccgtgaccggcacagcgtgccgtgtggcagaccccctaaaaaggctgtttaagcttggcaaacctctggcagcagacgatgaacatgatgatgacaggagaagggcattgcatgaagagtcaacacgctggaaccgagtgggtattctttcagagctgtgcaaggcagtagaatcaaggtatgaaaccgtaggaacttccatcatagttatggccatgactactctagctagcagtgttaaatcattcagctacctgagaggggcccctataactctctacggctaacctgaatggactacgacatagtctagtccgccaagtctagcatatgggcgcgccctcagcatcgattgaattggccaccatggtgagcaagggcgaggaggataacatggccatcatcaaggagttcatgcgcttcaaggtgcacatggagggctccgtgaacggccacgagttcgagatcgagggcgagggcgagggccgcccctacgagggcacccagaccgccaagctgaaggtgaccaagggtggccccctgcccttcgcctgggacatcctgtcccctcagttcatgtacggctccaaggcctacgtgaagcaccccgccgacatccccgactacttgaagctgtccttccccgagggcttcaagtgggagcgcgtgatgaacttcgaggacggcggcgtggtgaccgtgacccaggactcctccctgcaggacggcgagttcatctacaaggtgaagctgcgcggcaccaacttcccctccgacggccccgtaatgcagaagaagaccatgggctgggaggcctcctccgagcggatgtaccccgaggacggcgccctgaagggcgagatcaagcagaggctgaagctgaaggacggcggccactacgacgctgaggtcaagaccacctacaaggccaagaagcccgtgcagctgcccggcgcctacaacgtcaacatcaagttggacatcacctcccacaacgaggactacaccatcgtggaacagtacgaacgcgccgagggccgccactccaccggcggcatggacgagctgtacaagtaggaattggcaagctgcttacatagaactcgcggcgattggcatgccgccttaaaatttttattttatttttcttttcttttccgaatcggattttgtttttaatatttcaaaaaaaaaaaaaaaaaaaaaaaaaacgcgtcgaggggaattaattcttgaagacgaaagggccaggtggcacttttcggggaaatgtgcgcggaacccctatttgtttatttttctaaatacattcaaatatgtatccgctcatgagacaataaccctgataaatgcttcaataatattgaaaaaggaagagtatgagtattcaacatttccgtgtcgcccttattcccttttttgcggcattttgccttcctgtttttgctcacccagaaacgctggtgaaagtaaaagatgctgaagatcagttgggtgcacgagtgggttacatcgaactggatctcaacagcggtaagatccttgagagttttcgccccgaagaacgttttccaatgatgagcacttttaaagttctgctatgtggcgcggtattatcccgtgttgacgccgggcaagagcaactcggtcgccgcatacactattctcagaatgacttggttgagtactcaccagtcacagaaaagcatcttacggatggcatgacagtaagagaattatgcagtgctgccataaccatgagtgataacactgcggccaacttacttctgacaacgatcggaggaccgaaggagctaaccgcttttttgcacaacatgggggatcatgtaactcgccttgatcgttgggaaccggagctgaatgaagccataccaaacgacgagcgtgacaccacgatgcctgtagcaatggcaacaacgttgcgcaaactattaactggcgaactacttactctagcttcccggcaacaattaatagactggatggaggcggataaagttgcaggaccacttctgcgctcggcccttccggctggctggtttattgctgataaatctggagccggtgagcgtgggtctcgcggtatcattgcagcactggggccagatggtaagccctcccgtatcgtagttatctacacgacggggagtcaggcaactatggatgaacgaaatagacagatcgctgagataggtgcctcactgattaagcattggtaactgtcagaccaagtttactcatatatactttagattgatttaaaacttcatttttaatttaaaaggatctaggtgaagatcctttttgataatctcatgaccaaaatcccttaacgtgagttttcgttccactgagcgtcagaccccgtagaaaagatcaaaggatcttcttgagatcctttttttctgcgcgtaatctgctgcttgcaaacaaaaaaaccaccgctaccagcggtggtttgtttgccggatcaagagctaccaactctttttccgaaggtaactggcttcagcagagcgcagataccaaatactgtccttctagtgtagccgtagttaggccaccacttcaagaactctgtagcaccgcctacatacctcgctctgctaatcctgttaccagtggctgctgccagtggcgataagtcgtgtcttaccgggttggactcaagacgatagttaccggataaggcgcagcggtcgggctgaacggggggttcgtgcacacagcccagcttggagcgaacgacctacaccgaactgagatacctacagcgtgagcattgagaaagcgccacgcttcccgaagggagaaaggcggacaggtatccggtaagcggcagggtcggaacaggagagcgcacgagggagcttccagggggaaacgcctggtatctttatagtcctgtcgggtttcgccacctctgacttgagcgtcgatttttgtgatgctcgtcaggggggcggagcctatggaaaaacgccagcaacgcgagctctaatacgactcactatag

SEQ ID NO: 3 - DNA, 1629 bp, Artificial Sequence
  Synthetic polynucleotide
atgagggtccccgctcagctcctggggctcctgctgctctggctcccaggtgcacgatgtgccatgtgggagctggagaaagacgtttatgttgtagaggtggactggactcccgatgcccctggagaaacagtgaacctcacctgtgacacgcctgaagaagatgacatcacctggacctcagaccagagacatggagtcataggctctggaaagaccctgaccatcactgtcaaagagtttctagatgctggccagtacacctgccacaaaggaggcgagactctgagccactcacatctgctgctccacaagaaggaaaatggaatttggtccactgaaattttaaaaaatttcaaaaacaagactttcctgaagtgtgaagcaccaaattactccggacggttcacgtgctcatggctggtgcaaagaaacatggacttgaagttcaacatcaagagcagtagcagttcccctgactctcgggcagtgacatgtggaatggcgtctctgtctgcagagaaggtcacactggaccaaagggactatgagaagtattcagtgtcctgccaggaggatgtcacctgcccaactgccgaggagaccctgcccattgaactggcgttggaagcacggcagcagaataaatatgagaactacagcaccagcttcttcatcagggacatcatcaaaccagacccgcccaagaacttgcagatgaagcctttgaagaactcacaggtggaggtcagctgggagtaccctgactcctggagcactccccattcctacttctccctcaagttctttgttcgaatccagcgcaagaaagaaaagatgaaggagacagaggaggggtgtaaccagaaaggtgcgttcctcgtagagaagacatctaccgaagtccaatgcaaaggcgggaatgtctgcgtgcaagctcaggatcgctattacaattcctcatgcagcaagtgggcatgtgttccctgcagggtccgatccggaggttccggtggtggatccggaggtggctccggcggcggatccagggtcattccagtctctggacctgccaggtgtcttagccagtcccgaaacctgctgaagaccacagatgacatggtgaagacggccagagaaaaactgaaacattattcctgcactgctgaagacatcgatcatgaagacatcacacgggaccaaaccagcacattgaagacctgtttaccactggaactacacaagaacgagagttgcctggctactagagagacttcttccacaacaagagggagctgcctgcccccacagaagacgtctttgatgatgaccctgtgccttggtagcatctatgaggacttgaagatgtaccagacagagttccaggccatcaacgcagcacttcagaatcacaaccatcagcagatcattctagacaagggcatgctggtggccatcgatgagctgatgcagtctctgaatcataatggcgagactctgcgccagaaacctcctgtgggagaagcagacccttacagagtgaaaatgaagctctgcatcctgcttcacgccttcagcacccgcgtcgtgaccatcaacagggtgatgggctatctgagctccgcctga

SEQ ID NO: 4 - DNA, 12985 bp, Artificial Sequence
  Synthetic polynucleotide
atgggcggcgcatgagagaagcccagaccaattacctacccaaaatggagaaagttcacgttgacatcgaggaagacagcccattcctcagagctttgcagcggagcttcccgcagtttgaggtagaagccaagcaggtcactgataatgaccatgctaatgccagagcgttttcgcatctggcttcaaaactgatcgaaacggaggtggacccatccgacacgatccttgacattggaagtgcgcccgcccgcagaatgtattctaagcacaagtatcattgtatctgtccgatgagatgtgcggaagatccggacagattgtataagtatgcaactaagctgaagaaaaactgtaaggaaataactgataaggaattggacaagaaaatgaaggagctggccgccgtcatgagcgaccctgacctggaaactgagactatgtgcctccacgacgacgagtcgtgtcgctacgaagggcaagtcgctgtttaccaggatgtatacgcggttgacggaccgacaagtctctatcaccaagccaataagggagttagagtcgcctactggataggctttgacaccaccccttttatgtttaagaacttggctggagcatatccatcatactctaccaactgggccgacgaaaccgtgttaacggctcgtaacataggcctatgcagctctgacgttatggagcggtcacgtagagggatgtccattcttagaaagaagtatttgaaaccatccaacaatgttctattctctgttggctcgaccatctaccacgagaagagggacttactgaggagctggcacctgccgtctgtatttcacttacgtggcaagcaaaattacacatgtcggtgtgagactatagttagttgcgacgggtacgtcgttaaaagaatagctatcagtccaggcctgtatgggaagccttcaggctatgctgctacgatgcaccgcgagggattcttgtgctgcaaagtgacagacacattgaacggggagagggtctcttttcccgtgtgcacgtatgtgccagctacattgtgtgaccaaatgactggcatactggcaacagatgtcagtgcggacgacgcgcaaaaactgctggttgggctcaaccagcgtatagtcgtcaacggtcgcacccagagaaacaccaataccatgaaaaattaccttttgcccgtagtggcccaggcatttgctaggtgggcaaaggaatataaggaagatcaagaagatgaaaggccactaggactacgagatagacagttagtcatggggtgttgttgggcttttagaaggcacaagataacatctatttataagcgcccggatacccaaaccatcatcaaagtgaacagcgatttccactcattcgtgctgcccaggataggcagtaacacattggagatcgggctgagaacaagaatcaggaaaatgttagaggagcacaaggagccgtcacctctcattaccgccgaggacgtacaagaagctaagtgcgcagccgatgaggctaaggaggtgcgtgaagccgaggagttgcgcgcagctctaccacctttggcagctgatgttgaggagcccactctggaagccgatgtcgacttgatgttacaagaggctggggccggctcagtggagacacctcgtggcttgataaaggttaccagctacgatggcgaggacaagatcggctcttacgctgtgctttctccgcaggctgtactcaagagtgaaaaattatcttgcatccaccctctcgctgaacaagtcatagtgataacacactctggccgaaaagggcgttatgccgtggaaccataccatggtaaagtagtggtgccagagggacatgcaatacccgtccaggactttcaagctctgagtgaaagtgccaccattgtgtacaacgaacgtgagttcgtaaacaggtacctgcaccatattgccacacatggaggagcgctgaacactgatgaagaatattacaaaactgtcaagcccagcgagcacgacggcgaatacctgtacgacatcgacaggaaacagtgcgtcaagaaagaactagtcactgggctagggctcacaggcgagctggtggatcctcccttccatgaattcgcctacgagagtctgagaacacgaccagccgctccttaccaagtaccaaccataggggtgtatggcgtgccaggatcaggcaagtctggcatcattaaaagcgcagtcaccaaaaaagatctagtggtgagcgccaagaaagaaaactgtgcagaaattataagggacgtcaagaaaatgaaagggctggacgtcaatgccagaactgtggactcagtgctcttgaatggatgcaaacaccccgtagagaccctgtatattgacgaagcttttgcttgtcatgcaggtactctcagagcgctcatagccattataagacctaaaaaggcagtgctctgcggggatcccaaacagtgcggtttttttaacatgatgtgcctgaaagtgcattttaaccacgagatttgcacacaagtcttccacaaaagcatctctcgccgttgcactaaatctgtgacttcggtcgtctcaaccttgttttacgacaaaaaaatgagaacgacgaatccgaaagagactaagattgtgattgacactaccggcagtaccaaacctaagcaggacgatctcattctcacttgtttcagagggtgggtgaagcagttgcaaatagattacaaaggcaacgaaataatgacggcagctgcctctcaagggctgacccgtaaaggtgtgtatgccgttcggtacaaggtgaatgaaaatcctctgtacgcacccacctcagaacatgtgaacgtcctactgacccgcacggaggaccgcatcgtgtggaaaacactagccggcgacccatggataaaaacactgactgccaagtaccctgggaatttcactgccacgatagaggagtggcaagcagagcatgatgccatcatgaggcacatcttggagagaccggaccctaccgacgtcttccagaataaggcaaacgtgtgttgggccaaggctttagtgccggtgctgaagaccgctggcatagacatgaccactgaacaatggaacactgtggattattttgaaacggacaaagctcactcagcagagatagtattgaaccaactatgcgtgaggttctttggactcgatctggactccggtctattttctgcacccactgttccgttatccattaggaataatcactgggataactccccgtcgcctaacatgtacgggctgaataaagaagtggtccgtcagctctctcgcaggtacccacaactgcctcgggcagttgccactggaagagtctatgacatgaacactggtacactgcgcaattatgatccgcgcataaacctagtacctgtaaacagaagactgcctcatgctttagtcctccaccataatgaacacccacagagtgacttttcttcattcgtcagcaaattgaagggcagaactgtcctggtggtcggggaaaagttgtccgtcccaggcaaaatggttgactggttgtcagaccggcctgaggctaccttcagagctcggctggatttaggcatcccaggtgatgtgcccaaatatgacataatatttgttaatgtgaggaccccatataaataccatcactatcagcagtgtgaagaccatgccattaagcttagcatgttgaccaagaaagcttgtctgcatctgaatcccggcggaacctgtgtcagcataggttatggttacgctgacagggccagcgaaagcatcattggtgctatagcgcggcagttcaagttttcccgggtatgcaaaccgaaatcctcacttgaagagacggaagttctgtttgtattcattcggtacgatcgcaaggcccgtacgcacaattcttacaagctttcatcaaccttgaccaacatttatacaggttccagactccacgaagccggatgtgcaccctcatatcatgtggtgcgaggggatattgccacggccaccgaaggagtgattataaatgctgctaacagcaaaggacaacctggcggaggggtgtgcggagcgctgtataagaaattcccggaaagcttcgatttacagccgatcgaagtaggaaaagcgcgactggtcaaaggtgcagctaaacatatcattcatgccgtaggaccaaacttcaacaaagtttcggaggttgaaggtgacaaacagttggcagaggcttatgagtccatcgctaagattgtcaacgataacaattacaagtcagtagcgattccactgttgtccaccggcatcttttccgggaacaaagatcgactaacccaatcattgaaccatttgctgacagctttagacaccactgatgcagatgtagccatatactgcagggacaagaaatgggaaatgactctcaaggaagcagtggctaggagagaagcagtggaggagatatgcatatccgacgactcttcagtgacagaacctgatgcagagctggtgagggtgcatccgaagagttctttggctggaaggaagggctacagcacaagcgatggcaaaactttctcatatttggaagggaccaagtttcaccaggcggccaaggatatagcagaaattaatgccatgtggcccgttgcaacggaggccaatgagcaggtatgcatgtatatcctcggagaaggcatgagcagtattaggtcgaaatgccccgtcgaagagtcggaagcctccacaccacctagcacgctgccttgcttgtgcatccatgccatgactccagaaagagtacagcgcctaaaagcctcacgtccagaacaaattactgtgtgctcatcctttccattgccgaagtatagaatcactggtgtgcagaagatccaatgctcccagcctatattgttctcaccgaaagtgcctgcgtatattcatccaaggaagtatctcgtggaaacaccaccggtagacgagactccggagccatcggcagagaaccaatccacagaggggacacctgaacaaccaccacttataaccgaggatgagaccaggactagaacgcctgagccgatcatcatcgaagaggaagaagaggatagcataagtttgctgtcagatggcccgacccaccaggtgctgcaagtcgaggcagacattcacgggccgccctctgtatctagctcatcctggtccattcctcatgcatccgactttgatgtggacagtttatccatacttgacaccctggagggagctagcgtgaccagcggggcaacgtcagccgagactaactcttacttcgcaaagagtatggagtttctggcgcgaccggtgcctgcgcctcgaacagtattcaggaaccctccacatcccgctccgcgcacaagaacaccgtcacttgcacccagcagggcctgctcgagaaccagcctagtttccaccccgccaggcgtgaatagggtgatcactagagaggagctcgaggcgcttaccccgtcacgcactcctagcaggtcggtctcgagaaccagcctggtctccaacccgccaggcgtaaatagggtgattacaagagaggagtttgaggcgttcgtagcacaacaacaatgacggtttgatgcgggtgcatacatcttttcctccgacaccggtcaagggcatttacaacaaaaatcagtaaggcaaacggtgctatccgaagtggtgttggagaggaccgaattggagatttcgtatgccccgcgcctcgaccaagaaaaagaagaattactacgcaagaaattacagttaaatcccacacctgctaacagaagcagataccagtccaggaaggtggagaacatgaaagccataacagctagacgtattctgcaaggcctagggcattatttgaaggcagaaggaaaagtggagtgctaccgaaccctgcatcctgttcctttgtattcatctagtgtgaaccgtgccttttcaagccccaaggtcgcagtggaagcctgtaacgccatgttgaaagagaactttccgactgtggcttcttactgtattattccagagtacgatgcctatttggacatggttgacggagcttcatgctgcttagacactgccagtttttgccctgcaaagctgcgcagctttccaaagaaacactcctatttggaacccacaatacgatcggcagtgccttcagcgatccagaacacgctccagaacgtcctggcagctgccacaaaaagaaattgcaatgtcacgcaaatgagagaattgcccgtattggattcggcggcctttaatgtggaatgcttcaagaaatatgcgtgtaataatgaatattgggaaacgtttaaagaaaaccccatcaggcttactgaagaaaacgtggtaaattacattaccaaattaaaaggaccaaaagctgctgctctttttgcgaagacacataatttgaatatgttgcaggacataccaatggacaggtttgtaatggacttaaagagagacgtgaaagtgactccaggaacaaaacatactgaagaacggcccaaggtacaggtgatccaggctgccgatccgctagcaacagcgtatctgtgcggaatccaccgagagctggttaggagattaaatgcggtcctgcttccgaacattcatacactgtttgatatgtcggctgaagactttgacgctattatagccgagcacttccagcctggggattgtgttctggaaactgacatcgcgtcgtttgataaaagtgaggacgacgccatggctctgaccgcgttaatgattctggaagacttaggtgtggacgcagagctgttgacgctgattgaggcggctttcggcgaaatttcatcaatacatttgcccactaaaactaaatttaaattcggagccatgatgaaatctggaatgttcctcacactgtttgtgaacacagtcattaacattgtaatcgcaagcagagtgttgagagaacggctaaccggatcaccatgtgcagcattcattggagatgacaatatcgtgaaaggagtcaaatcggacaaattaatggcagacaggtgcgccacctggttgaatatggaagtcaagattatagatgctgtggtgggcgagaaagcgccttatttctgtggagggtttattttgtgtgactccgtgaccggcacagcgtgccgtgtggcagaccccctaaaaaggctgtttaagcttggcaaacctctggcagcagacgatgaacatgatgatgacaggagaagggcattgcatgaagagtcaacacgctggaaccgagtgggtattctttcagagctgtgcaaggcagtagaatcaaggtatgaaaccgtaggaacttccatcatagttatggccatgactactctagctagcagtgttaaatcattcagctacctgagaggggcccctataactctctacggctaacctgaatggactacgacatagtctagtccgccaagtctagcatatgggcgcgccctcagcatcgatttgaattggccaccatgagggtccccgctcagctcctggggctcctgctgctctggctcccaggtgcacgatgtgccatgtgggagctggagaaagacgtttatgttgtagaggtggactggactcccgatgcccctggagaaacagtgaacctcacctgtgacacgcctgaagaagatgacatcacctggacctcagaccagagacatggagtcataggctctggaaagaccctgaccatcactgtcaaagagtttctagatgctggccagtacacctgccacaaaggaggcgagactctgagccactcacatctgctgctccacaagaaggaaaatggaatttggtccactgaaattttaaaaaatttcaaaaacaagactttcctgaagtgtgaagcaccaaattactccggacggttcacgtgctcatggctggtgcaaagaaacatggacttgaagttcaacatcaagagcagtagcagttcccctgactctcgggcagtgacatgtggaatggcgtctctgtctgcagagaaggtcacactggaccaaagggactatgagaagtattcagtgtcctgccaggaggatgtcacctgcccaactgccgaggagaccctgcccattgaactggcgttggaagcacggcagcagaataaatatgagaactacagcaccagcttcttcatcagggacatcatcaaaccagacccgcccaagaacttgcagatgaagcctttgaagaactcacaggtggaggtcagctgggagtaccctgactcctggagcactccccattcctacttctccctcaagttctttgttcgaatccagcgcaagaaagaaaagatgaaggagacagaggaggggtgtaaccagaaaggtgcgttcctcgtagagaagacatctaccgaagtccaatgcaaaggcgggaatgtctgcgtgcaagctcaggatcgctattacaattcctcatgcagcaagtgggcatgtgttccctgcagggtccgatccggaggttccggtggtggatccggaggtggctccggcggcggatccagggtcattccagtctctggacctgccaggtgtcttagccagtcccgaaacctgctgaagaccacagatgacatggtgaagacggccagagaaaaactgaaacattattcctgcactgctgaagacatcgatcatgaagacatcacacgggaccaaaccagcacattgaagacctgtttaccactggaactacacaagaacgagagttgcctggctactagagagacttcttccacaacaagagggagctgcctgcccccacagaagacgtctttgatgatgaccctgtgccttggtagcatctatgaggacttgaagatgtaccagacagagttccaggccatcaacgcagcacttcagaatcacaaccatcagcagatcattctagacaagggcatgctggtggccatcgatgagctgatgcagtctctgaatcataatggcgagactctgcgccagaaacctcctgtgggagaagcagacccttacagagtgaaaatgaagctctgcatcctgcttcacgccttcagcacccgcgtcgtgaccatcaacagggtgatgggctatctgagctccgccggttccggtggcggatccgaagcacacaagagtgagatcgcccatcggtataatgatttgggagaacaacatttcaaaggcctagtcctgattgccttttcccagtatctccagaaatgctcatacgatgagcatgccaaattagtgcaggaagtaacagactttgcaaagacgtgtgttgccgatgagtctgccgccaactgtgacaaatcccttcacactctttttggagataagttgtgtgccattccaaacctccgtgaaaactatggtgaactggctgactgctgtacaaaacaagagcccgaaagaaacgaatgtttcctgcaacacaaagatgacaaccccagcctgccaccatttgaaaggccagaggctgaggccatgtgcacctcctttaaggaaaacccaaccacctttatgggacactatttgcatgaagttgccagaagacatccttatttctatgccccagaacttctttactatgctgagcagtacaatgagattctgacccagtgttgtgcagaggctgacaaggaaagctgcctgaccccgaagcttgatggtgtgaaggagaaagcattggtctcatctgtccgtcagagaatgaagtgctccagtatgcagaagtttggagagagagcttttaaagcatgggcagtagctcgtctgagccagacattccccaatgctgactttgcagaaatcaccaaattggcaacagacctgaccaaagtcaacaaggagtgctgccatggtgacctgctggaatgcgcagatgacagggcggaacttgccaagtacatgtgtgaaaaccaggcgactatctccagcaaactgcagacttgctgcgataaaccactgttgaagaaagcccactgtcttagtgaggtggagcatgacaccatgcctgctgatctgcctgccattgctgctgattttgttgaggaccaggaagtgtgcaagaactatgctgaggccaaggatgtcttcctgggcacgttcttgtatgaatattcaagaagacaccctgattactctgtatccctgttgctgagacttgctaagaaatatgaagccactctggaaaagtgctgcgctgaagccaatcctcccgcatgctacggcacagtgcttgctgaatttcagcctcttgtagaagagcctaagaacttggtcaaaaccaactgtgatctttacgagaagcttggagaatatggattccaaaatgccattctagttcgctacacccagaaagcacctcaggtgtcaaccccaactctcgtggaggctgcaagaaacctaggaagagtgggcaccaagtgttgtacacttcctgaagatcagagactgccttgtgtggaagactatctgtctgcaatcctgaaccgtgtgtgtctgctgcatgagaagaccccagtgagtgagcatgttaccaagtgctgtagtggatccctggtggaaaggcggccatgcttctctgctctgacagttgatgaaacatatgtccccaaagagtttaaagctgagaccttcaccttccactctgatatctgcacacttccagagaaggagaagcagattaagaaacaaacggctcttgctgagctggtgaagcacaagcccaaggctacagcggagcaactgaagactgtcatggatgactttgcacagttcctggatacatgttgcaaggctgctgacaaggacacctgcttctcgactgagggtccaaaccttgtcactagatgcaaagacgccttagcctgagcgatcgctaaatacagcagcaattggcaagctgcttacatagaactcgcggcgattggcatgccgccttaaaatttttattttatttttcttttcttttccgaatcggattttgtttttaatatttcaaaaaaaaaaaaaaaaaaaaaaaaaacgcgtcgaggggaattaattcttgaagacgaaagggccaggtggcacttttcggggaaatgtgcgcggaacccctatttgtttatttttctaaatacattcaaatatgtatccgctcatgagacaataaccctgataaatgcttcaataatattgaaaaaggaagagtatgagtattcaacatttccgtgtcgcccttattcccttttttgcggcattttgccttcctgtttttgctcacccagaaacgctggtgaaagtaaaagatgctgaagatcagttgggtgcacgagtgggttacatcgaactggatctcaacagcggtaagatccttgagagttttcgccccgaagaacgttttccaatgatgagcacttttaaagttctgctatgtggcgcggtattatcccgtgttgacgccgggcaagagcaactcggtcgccgcatacactattctcagaatgacttggttgagtactcaccagtcacagaaaagcatcttacggatggcatgacagtaagagaattatgcagtgctgccataaccatgagtgataacactgcggccaacttacttctgacaacgatcggaggaccgaaggagctaaccgcttttttgcacaacatgggggatcatgtaactcgccttgatcgttgggaaccggagctgaatgaagccataccaaacgacgagcgtgacaccacgatgcctgtagcaatggcaacaacgttgcgcaaactattaactggcgaactacttactctagcttcccggcaacaattaatagactggatggaggcggataaagttgcaggaccacttctgcgctcggcccttccggctggctggtttattgctgataaatctggagccggtgagcgtgggtctcgcggtatcattgcagcactggggccagatggtaagccctcccgtatcgtagttatctacacgacggggagtcaggcaactatggatgaacgaaatagacagatcgctgagataggtgcctcactgattaagcattggtaactgtcagaccaagtttactcatatatactttagattgatttaaaacttcatttttaatttaaaaggatctaggtgaagatcctttttgataatctcatgaccaaaatcccttaacgtgagttttcgttccactgagcgtcagaccccgtagaaaagatcaaaggatcttcttgagatcctttttttctgcgcgtaatctgctgcttgcaaacaaaaaaaccaccgctaccagcggtggtttgtttgccggatcaagagctaccaactctttttccgaaggtaactggcttcagcagagcgcagataccaaatactgtccttctagtgtagccgtagttaggccaccacttcaagaactctgtagcaccgcctacatacctcgctctgctaatcctgttaccagtggctgctgccagtggcgataagtcgtgtcttaccgggttggactcaagacgatagttaccggataaggcgcagcggtcgggctgaacggggggttcgtgcacacagcccagcttggagcgaacgacctacaccgaactgagatacctacagcgtgagcattgagaaagcgccacgcttcccgaagggagaaaggcggacaggtatccggtaagcggcagggtcggaacaggagagcgcacgagggagcttccagggggaaacgcctggtatctttatagtcctgtcgggtttcgccacctctgacttgagcgtcgatttttgtgatgctcgtcaggggggcggagcctatggaaaaacgccagcaacgcgagctctaatacgactcactatag

SEQ ID NO: 5 - DNA, 13981 bp, Artificial Sequence
  Synthetic polynucleotide
atgggcggcgcatgagagaagcccagaccaattacctacccaaaatggagaaagttcacgttgacatcgaggaagacagcccattcctcagagctttgcagcggagcttcccgcagtttgaggtagaagccaagcaggtcactgataatgaccatgctaatgccagagcgttttcgcatctggcttcaaaactgatcgaaacggaggtggacccatccgacacgatccttgacattggaagtgcgcccgcccgcagaatgtattctaagcacaagtatcattgtatctgtccgatgagatgtgcggaagatccggacagattgtataagtatgcaactaagctgaagaaaaactgtaaggaaataactgataaggaattggacaagaaaatgaaggagctggccgccgtcatgagcgaccctgacctggaaactgagactatgtgcctccacgacgacgagtcgtgtcgctacgaagggcaagtcgctgtttaccaggatgtatacgcggttgacggaccgacaagtctctatcaccaagccaataagggagttagagtcgcctactggataggctttgacaccaccccttttatgtttaagaacttggctggagcatatccatcatactctaccaactgggccgacgaaaccgtgttaacggctcgtaacataggcctatgcagctctgacgttatggagcggtcacgtagagggatgtccattcttagaaagaagtatttgaaaccatccaacaatgttctattctctgttggctcgaccatctaccacgagaagagggacttactgaggagctggcacctgccgtctgtatttcacttacgtggcaagcaaaattacacatgtcggtgtgagactatagttagttgcgacgggtacgtcgttaaaagaatagctatcagtccaggcctgtatgggaagccttcaggctatgctgctacgatgcaccgcgagggattcttgtgctgcaaagtgacagacacattgaacggggagagggtctcttttcccgtgtgcacgtatgtgccagctacattgtgtgaccaaatgactggcatactggcaacagatgtcagtgcggacgacgcgcaaaaactgctggttgggctcaaccagcgtatagtcgtcaacggtcgcacccagagaaacaccaataccatgaaaaattaccttttgcccgtagtggcccaggcatttgctaggtgggcaaaggaatataaggaagatcaagaagatgaaaggccactaggactacgagatagacagttagtcatggggtgttgttgggcttttagaaggcacaagataacatctatttataagcgcccggatacccaaaccatcatcaaagtgaacagcgatttccactcattcgtgctgcccaggataggcagtaacacattggagatcgggctgagaacaagaatcaggaaaatgttagaggagcacaaggagccgtcacctctcattaccgccgaggacgtacaagaagctaagtgcgcagccgatgaggctaaggaggtgcgtgaagccgaggagttgcgcgcagctctaccacctttggcagctgatgttgaggagcccactctggaagccgatgtcgacttgatgttacaagaggctggggccggctcagtggagacacctcgtggcttgataaaggttaccagctacgatggcgaggacaagatcggctcttacgctgtgctttctccgcaggctgtactcaagagtgaaaaattatcttgcatccaccctctcgctgaacaagtcatagtgataacacactctggccgaaaagggcgttatgccgtggaaccataccatggtaaagtagtggtgccagagggacatgcaatacccgtccaggactttcaagctctgagtgaaagtgccaccattgtgtacaacgaacgtgagttcgtaaacaggtacctgcaccatattgccacacatggaggagcgctgaacactgatgaagaatattacaaaactgtcaagcccagcgagcacgacggcgaatacctgtacgacatcgacaggaaacagtgcgtcaagaaagaactagtcactgggctagggctcacaggcgagctggtggatcctcccttccatgaattcgcctacgagagtctgagaacacgaccagccgctccttaccaagtaccaaccataggggtgtatggcgtgccaggatcaggcaagtctggcatcattaaaagcgcagtcaccaaaaaagatctagtggtgagcgccaagaaagaaaactgtgcagaaattataagggacgtcaagaaaatgaaagggctggacgtcaatgccagaactgtggactcagtgctcttgaatggatgcaaacaccccgtagagaccctgtatattgacgaagcttttgcttgtcatgcaggtactctcagagcgctcatagccattataagacctaaaaaggcagtgctctgcggggatcccaaacagtgcggtttttttaacatgatgtgcctgaaagtgcattttaaccacgagatttgcacacaagtcttccacaaaagcatctctcgccgttgcactaaatctgtgacttcggtcgtctcaaccttgttttacgacaaaaaaatgagaacgacgaatccgaaagagactaagattgtgattgacactaccggcagtaccaaacctaagcaggacgatctcattctcacttgtttcagagggtgggtgaagcagttgcaaatagattacaaaggcaacgaaataatgacggcagctgcctctcaagggctgacccgtaaaggtgtgtatgccgttcggtacaaggtgaatgaaaatcctctgtacgcacccacctcagaacatgtgaacgtcctactgacccgcacggaggaccgcatcgtgtggaaaacactagccggcgacccatggataaaaacactgactgccaagtaccctgggaatttcactgccacgatagaggagtggcaagcagagcatgatgccatcatgaggcacatcttggagagaccggaccctaccgacgtcttccagaataaggcaaacgtgtgttgggccaaggctttagtgccggtgctgaagaccgctggcatagacatgaccactgaacaatggaacactgtggattattttgaaacggacaaagctcactcagcagagatagtattgaaccaactatgcgtgaggttctttggactcgatctggactccggtctattttctgcacccactgttccgttatccattaggaataatcactgggataactccccgtcgcctaacatgtacgggctgaataaagaagtggtccgtcagctctctcgcaggtacccacaactgcctcgggcagttgccactggaagagtctatgacatgaacactggtacactgcgcaattatgatccgcgcataaacctagtacctgtaaacagaagactgcctcatgctttagtcctccaccataatgaacacccacagagtgacttttcttcattcgtcagcaaattgaagggcagaactgtcctggtggtcggggaaaagttgtccgtcccaggcaaaatggttgactggttgtcagaccggcctgaggctaccttcagagctcggctggatttaggcatcccaggtgatgtgcccaaatatgacataatatttgttaatgtgaggaccccatataaataccatcactatcagcagtgtgaagaccatgccattaagcttagcatgttgaccaagaaagcttgtctgcatctgaatcccggcggaacctgtgtcagcataggttatggttacgctgacagggccagcgaaagcatcattggtgctatagcgcggcagttcaagttttcccgggtatgcaaaccgaaatcctcacttgaagagacggaagttctgtttgtattcattcggtacgatcgcaaggcccgtacgcacaattcttacaagctttcatcaaccttgaccaacatttatacaggttccagactccacgaagccggatgtgcaccctcatatcatgtggtgcgaggggatattgccacggccaccgaaggagtgattataaatgctgctaacagcaaaggacaacctggcggaggggtgtgcggagcgctgtataagaaattcccggaaagcttcgatttacagccgatcgaagtaggaaaagcgcgactggtcaaaggtgcagctaaacatatcattcatgccgtaggaccaaacttcaacaaagtttcggaggttgaaggtgacaaacagttggcagaggcttatgagtccatcgctaagattgtcaacgataacaattacaagtcagtagcgattccactgttgtccaccggcatcttttccgggaacaaagatcgactaacccaatcattgaaccatttgctgacagctttagacaccactgatgcagatgtagccatatactgcagggacaagaaatgggaaatgactctcaaggaagcagtggctaggagagaagcagtggaggagatatgcatatccgacgactcttcagtgacagaacctgatgcagagctggtgagggtgcatccgaagagttctttggctggaaggaagggctacagcacaagcgatggcaaaactttctcatatttggaagggaccaagtttcaccaggcggccaaggatatagcagaaattaatgccatgtggcccgttgcaacggaggccaatgagcaggtatgcatgtatatcctcggagaaggcatgagcagtattaggtcgaaatgccccgtcgaagagtcggaagcctccacaccacctagcacgctgccttgcttgtgcatccatgccatgactccagaaagagtacagcgcctaaaagcctcacgtccagaacaaattactgtgtgctcatcctttccattgccgaagtatagaatcactggtgtgcagaagatccaatgctcccagcctatattgttctcaccgaaagtgcctgcgtatattcatccaaggaagtatctcgtggaaacaccaccggtagacgagactccggagccatcggcagagaaccaatccacagaggggacacctgaacaaccaccacttataaccgaggatgagaccaggactagaacgcctgagccgatcatcatcgaagaggaagaagaggatagcataagtttgctgtcagatggcccgacccaccaggtgctgcaagtcgaggcagacattcacgggccgccctctgtatctagctcatcctggtccattcctcatgcatccgactttgatgtggacagtttatccatacttgacaccctggagggagctagcgtgaccagcggggcaacgtcagccgagactaactcttacttcgcaaagagtatggagtttctggcgcgaccggtgcctgcgcctcgaacagtattcaggaaccctccacatcccgctccgcgcacaagaacaccgtcacttgcacccagcagggcctgctcgagaaccagcctagtttccaccccgccaggcgtgaatagggtgatcactagagaggagctcgaggcgcttaccccgtcacgcactcctagcaggtcggtctcgagaaccagcctggtctccaacccgccaggcgtaaatagggtgattacaagagaggagtttgaggcgttcgtagcacaacaacaatgacggtttgatgcgggtgcatacatcttttcctccgacaccggtcaagggcatttacaacaaaaatcagtaaggcaaacggtgctatccgaagtggtgttggagaggaccgaattggagatttcgtatgccccgcgcctcgaccaagaaaaagaagaattactacgcaagaaattacagttaaatcccacacctgctaacagaagcagataccagtccaggaaggtggagaacatgaaagccataacagctagacgtattctgcaaggcctagggcattatttgaaggcagaaggaaaagtggagtgctaccgaaccctgcatcctgttcctttgtattcatctagtgtgaaccgtgccttttcaagccccaaggtcgcagtggaagcctgtaacgccatgttgaaagagaactttccgactgtggcttcttactgtattattccagagtacgatgcctatttggacatggttgacggagcttcatgctgcttagacactgccagtttttgccctgcaaagctgcgcagctttccaaagaaacactcctatttggaacccacaatacgatcggcagtgccttcagcgatccagaacacgctccagaacgtcctggcagctgccacaaaaagaaattgcaatgtcacgcaaatgagagaattgcccgtattggattcggcggcctttaatgtggaatgcttcaagaaatatgcgtgtaataatgaatattgggaaacgtttaaagaaaaccccatcaggcttactgaagaaaacgtggtaaattacattaccaaattaaaaggaccaaaagctgctgctctttttgcgaagacacataatttgaatatgttgcaggacataccaatggacaggtttgtaatggacttaaagagagacgtgaaagtgactccaggaacaaaacatactgaagaacggcccaaggtacaggtgatccaggctgccgatccgctagcaacagcgtatctgtgcggaatccaccgagagctggttaggagattaaatgcggtcctgcttccgaacattcatacactgtttgatatgtcggctgaagactttgacgctattatagccgagcacttccagcctggggattgtgttctggaaactgacatcgcgtcgtttgataaaagtgaggacgacgccatggctctgaccgcgttaatgattctggaagacttaggtgtggacgcagagctgttgacgctgattgaggcggctttcggcgaaatttcatcaatacatttgcccactaaaactaaatttaaattcggagccatgatgaaatctggaatgttcctcacactgtttgtgaacacagtcattaacattgtaatcgcaagcagagtgttgagagaacggctaaccggatcaccatgtgcagcattcattggagatgacaatatcgtgaaaggagtcaaatcggacaaattaatggcagacaggtgcgccacctggttgaatatggaagtcaagattatagatgctgtggtgggcgagaaagcgccttatttctgtggagggtttattttgtgtgactccgtgaccggcacagcgtgccgtgtggcagaccccctaaaaaggctgtttaagcttggcaaacctctggcagcagacgatgaacatgatgatgacaggagaagggcattgcatgaagagtcaacacgctggaaccgagtgggtattctttcagagctgtgcaaggcagtagaatcaaggtatgaaaccgtaggaacttccatcatagttatggccatgactactctagctagcagtgttaaatcattcagctacctgagaggggcccctataactctctacggctaacctgaatggactacgacatagtctagtccgccaagtctagcatatgggcgcgccctcagcatcgatttgaattggccaccatgagggtccccgctcagctcctggggctcctgctgctctggctcccaggtgcacgatgtgccatgtgggagctggagaaagacgtttatgttgtagaggtggactggactcccgatgcccctggagaaacagtgaacctcacctgtgacacgcctgaagaagatgacatcacctggacctcagaccagagacatggagtcataggctctggaaagaccctgaccatcactgtcaaagagtttctagatgctggccagtacacctgccacaaaggaggcgagactctgagccactcacatctgctgctccacaagaaggaaaatggaatttggtccactgaaattttaaaaaatttcaaaaacaagactttcctgaagtgtgaagcaccaaattactccggacggttcacgtgctcatggctggtgcaaagaaacatggacttgaagttcaacatcaagagcagtagcagttcccctgactctcgggcagtgacatgtggaatggcgtctctgtctgcagagaaggtcacactggaccaaagggactatgagaagtattcagtgtcctgccaggaggatgtcacctgcccaactgccgaggagaccctgcccattgaactggcgttggaagcacggcagcagaataaatatgagaactacagcaccagcttcttcatcagggacatcatcaaaccagacccgcccaagaacttgcagatgaagcctttgaagaactcacaggtggaggtcagctgggagtaccctgactcctggagcactccccattcctacttctccctcaagttctttgttcgaatccagcgcaagaaagaaaagatgaaggagacagaggaggggtgtaaccagaaaggtgcgttcctcgtagagaagacatctaccgaagtccaatgcaaaggcgggaatgtctgcgtgcaagctcaggatcgctattacaattcctcatgcagcaagtgggcatgtgttccctgcagggtccgatccggaggttccggtggtggatccggaggtggctccggcggcggatccagggtcattccagtctctggacctgccaggtgtcttagccagtcccgaaacctgctgaagaccacagatgacatggtgaagacggccagagaaaaactgaaacattattcctgcactgctgaagacatcgatcatgaagacatcacacgggaccaaaccagcacattgaagacctgtttaccactggaactacacaagaacgagagttgcctggctactagagagacttcttccacaacaagagggagctgcctgcccccacagaagacgtctttgatgatgaccctgtgccttggtagcatctatgaggacttgaagatgtaccagacagagttccaggccatcaacgcagcacttcagaatcacaaccatcagcagatcattctagacaagggcatgctggtggccatcgatgagctgatgcagtctctgaatcataatggcgagactctgcgccagaaacctcctgtgggagaagcagacccttacagagtgaaaatgaagctctgcatcctgcttcacgccttcagcacccgcgtcgtgaccatcaacagggtgatgggctatctgagctccgccggttccggtggcggatccgaagcacacaagagtgagatcgcccatcggtataatgatttgggagaacaacatttcaaaggcctagtcctgattgccttttcccagtatctccagaaatgctcatacgatgagcatgccaaattagtgcaggaagtaacagactttgcaaagacgtgtgttgccgatgagtctgccgccaactgtgacaaatcccttcacactctttttggagataagttgtgtgccattccaaacctccgtgaaaactatggtgaactggctgactgctgtacaaaacaagagcccgaaagaaacgaatgtttcctgcaacacaaagatgacaaccccagcctgccaccatttgaaaggccagaggctgaggccatgtgcacctcctttaaggaaaacccaaccacctttatgggacactatttgcatgaagttgccagaagacatccttatttctatgccccagaacttctttactatgctgagcagtacaatgagattctgacccagtgttgtgcagaggctgacaaggaaagctgcctgaccccgaagcttgatggtgtgaaggagaaagcattggtctcatctgtccgtcagagaatgaagtgctccagtatgcagaagtttggagagagagcttttaaagcatgggcagtagctcgtctgagccagacattccccaatgctgactttgcagaaatcaccaaattggcaacagacctgaccaaagtcaacaaggagtgctgccatggtgacctgctggaatgcgcagatgacagggcggaacttgccaagtacatgtgtgaaaaccaggcgactatctccagcaaactgcagacttgctgcgataaaccactgttgaagaaagcccactgtcttagtgaggtggagcatgacaccatgcctgctgatctgcctgccattgctgctgattttgttgaggaccaggaagtgtgcaagaactatgctgaggccaaggatgtcttcctgggcacgttcttgtatgaatattcaagaagacaccctgattactctgtatccctgttgctgagacttgctaagaaatatgaagccactctggaaaagtgctgcgctgaagccaatcctcccgcatgctacggcacagtgcttgctgaatttcagcctcttgtagaagagcctaagaacttggtcaaaaccaactgtgatctttacgagaagcttggagaatatggattccaaaatgccattctagttcgctacacccagaaagcacctcaggtgtcaaccccaactctcgtggaggctgcaagaaacctaggaagagtgggcaccaagtgttgtacacttcctgaagatcagagactgccttgtgtggaagactatctgtctgcaatcctgaaccgtgtgtgtctgctgcatgagaagaccccagtgagtgagcatgttaccaagtgctgtagtggatccctggtggaaaggcggccatgcttctctgctctgacagttgatgaaacatatgtccccaaagagtttaaagctgagaccttcaccttccactctgatatctgcacacttccagagaaggagaagcagattaagaaacaaacggctcttgctgagctggtgaagcacaagcccaaggctacagcggagcaactgaagactgtcatggatgactttgcacagttcctggatacatgttgcaaggctgctgacaaggacacctgcttctcgactgagggtccaaaccttgtcactagatgcaaagacgccttagccggcggaggttccggtggcggatcccaatactatgactacgatatacccctgttcatgtacgggcaaatatctccaaactgtgcaccagaatgtaactgccctcactcataccccactgcaatgtactgtgacgacctgaagttgaaatccgtgccaatggtgcctcctgggattaagtacctgtacctccgcaacaatcagatcgaccatattgacgagaaggcttttgaaaacgtcacagacctccagtggcttatcctggaccataacctgcttgaaaatagtaagataaagggcaaagtattttccaaacttaaacagcttaaaaaactccacatcaactacaataaccttactgaatccgtgggaccattgccaaaatctctccaagatttgcagttgactaacaacaagatatccaaactcggctccttcgatgggctggttaatctgactttcatctacttgcaacacaaccaattgaaggaggatgcagtttcagctagtcttaaaggtctgaaaagccttgagtatcttgatctgtcatttaatcaaatgtccaagctccctgctgggctcccaacaagtctgctgacactctatctcgacaataacaagataagtaacattcccgatgagtactttaaaagatttaccggcctccaatacttgcggctttctcacaacgagttggcagactctggtgtacccggcaactcctttaatataagttctcttctcgagcttgatttgtcctataacaaactgaagagtatccctactgtcaatgaaaatttggagaattactacctcgaagtcaatgagcttgagaagttcgatgttaagtctttctgtaagatactgggtccattgtcatacagcaagattaaacatcttcgcttggatgggaatcccttgactcaaagctcacttccccccgacatgtacgaatgcctgagggtagccaacgaaatcacagtaaacggaggtggctcctgagcgatcgctaaatacagcagcaattggcaagctgcttacatagaactcgcggcgattggcatgccgccttaaaatttttattttatttttcttttcttttccgaatcggattttgtttttaatatttcaaaaaaaaaaaaaaaaaaaaaaaaaacgcgtcgaggggaattaattcttgaagacgaaagggccaggtggcacttttcggggaaatgtgcgcggaacccctatttgtttatttttctaaatacattcaaatatgtatccgctcatgagacaataaccctgataaatgcttcaataatattgaaaaaggaagagtatgagtattcaacatttccgtgtcgcccttattcccttttttgcggcattttgccttcctgtttttgctcacccagaaacgctggtgaaagtaaaagatgctgaagatcagttgggtgcacgagtgggttacatcgaactggatctcaacagcggtaagatccttgagagttttcgccccgaagaacgttttccaatgatgagcacttttaaagttctgctatgtggcgcggtattatcccgtgttgacgccgggcaagagcaactcggtcgccgcatacactattctcagaatgacttggttgagtactcaccagtcacagaaaagcatcttacggatggcatgacagtaagagaattatgcagtgctgccataaccatgagtgataacactgcggccaacttacttctgacaacgatcggaggaccgaaggagctaaccgcttttttgcacaacatgggggatcatgtaactcgccttgatcgttgggaaccggagctgaatgaagccataccaaacgacgagcgtgacaccacgatgcctgtagcaatggcaacaacgttgcgcaaactattaactggcgaactacttactctagcttcccggcaacaattaatagactggatggaggcggataaagttgcaggaccacttctgcgctcggcccttccggctggctggtttattgctgataaatctggagccggtgagcgtgggtctcgcggtatcattgcagcactggggccagatggtaagccctcccgtatcgtagttatctacacgacggggagtcaggcaactatggatgaacgaaatagacagatcgctgagataggtgcctcactgattaagcattggtaactgtcagaccaagtttactcatatatactttagattgatttaaaacttcatttttaatttaaaaggatctaggtgaagatcctttttgataatctcatgaccaaaatcccttaacgtgagttttcgttccactgagcgtcagaccccgtagaaaagatcaaaggatcttcttgagatcctttttttctgcgcgtaatctgctgcttgcaaacaaaaaaaccaccgctaccagcggtggtttgtttgccggatcaagagctaccaactctttttccgaaggtaactggcttcagcagagcgcagataccaaatactgtccttctagtgtagccgtagttaggccaccacttcaagaactctgtagcaccgcctacatacctcgctctgctaatcctgttaccagtggctgctgccagtggcgataagtcgtgtcttaccgggttggactcaagacgatagttaccggataaggcgcagcggtcgggctgaacggggggttcgtgcacacagcccagcttggagcgaacgacctacaccgaactgagatacctacagcgtgagcattgagaaagcgccacgcttcccgaagggagaaaggcggacaggtatccggtaagcggcagggtcggaacaggagagcgcacgagggagcttccagggggaaacgcctggtatctttatagtcctgtcgggtttcgccacctctgacttgagcgtcgatttttgtgatgctcgtcaggggggcggagcctatggaaaaacgccagcaacgcgagctctaatacgactcactatag